European Patent Application EP 4 732 829 A1, published April 29, 2026. Title: GLP-1-Fc-FGF21双靶融合蛋白组合物和注射液及其用途. Applicant: 广东东阳光药业股份有限公司. Application CN. The sequence listing filed with the application follows.

SEQUENCE LISTING (12 sequences)

SEQ ID NO: 1 - protein, 470 aa, synthetic construct
HGEGTFTSDVSSYLEEQAAKEFIAWLVKGGGGGGGSGGGGSGGGGSESKYGPPCPPCPAPEAAGGPSVFLFPPKPKDTLMISRTPEVTCVVVDVSQEDPEVQFNWYVDGVEVHNAKTKPREEQFNSTYRVVSVLTVLHQDWLNGKEYKCKVSNKGLPSSIEKTISKAKGQPREPQVYTLPPSQEEMTKNQVSLTCLVKGFYPSDIAVEWESNGQPENNYKTTPPVLDSDGSFFLYSKLTVDKSRWQEGNVFSCSVMHEALHNHYTQKSLSLSLGGGGGSGGGGSGGGGSHPIPDSSPLLQFGGQVRQVYLYTDDAQQTEAHLEIREDGTVGGAADQSPESLLQLKALKPGVIQILGVKTSRFLCQRPDGALYGSLHFDPEACSFRERLLEDGYNVYQSEAHGLPLHLPGNKSPHRDPAPRGPARFLPLPGLPPALPEPPGILAPQPPDVGSSDPLHMVGASQGLSPSYAS

SEQ ID NO: 2 - protein, 470 aa, synthetic construct
HGEGTFTSDVSSYLEEQAAKEFIAWLVKGGGGGGGSGGGGSGGGGSESKYGPPCPPCPAPEAAGGPSVFLFPPKPKDTLMISRTPEVTCVVVDVSQEDPEVQFNWYVDGVEVHNAKTKPREEQFNSTYRVVSVLTVLHQDWLNGKEYKCKVSNKGLPSSIEKTISKAKGQPREPQVYTLPPSQEEMTKNQVSLTCLVKGFYPSDIAVEWESNGQPENNYKTTPPVLDSDGSFFLYSKLTVDKSRWQEGNVFSCSVMHEALHNHYTQKSLSLSLGGGGGSGGGGSGGGGSHPIPDSSPLLQFGGQVRQVYLYTDDAQQTEAHLEIREDGTVGGAADQSPESLLQLKALKPGVIQILGVKTSRFLCQRPDGALYGSLHFDPEACSFRERLLEDGYNVYQSEAHGLPLHLPGNKSPHRDPAPRGPARFLPLPGLPPALPEPPGILAPQPPDVGSSDPLHMVGGSQGLSPSYAS

SEQ ID NO: 3 - protein, 470 aa, synthetic construct
HGEGTFTSDVSSYLEEQAAKEFIAWLVKGGGGGGGSGGGGSGGGGSESKYGPPCPPCPAPEAAGGPSVFLFPPKPKDTLMISRTPEVTCVVVDVSQEDPEVQFNWYVDGVEVHNAKTKPREEQFNSTYRVVSVLTVLHQDWLNGKEYKCKVSNKGLPSSIEKTISKAKGQPREPQVYTLPPSQEEMTKNQVSLTCLVKGFYPSDIAVEWESNGQPENNYKTTPPVLDSDGSFFLYSKLTVDKSRWQEGNVFSCSVMHEALHNHYTQKSLSLSLGGGGGSGGGGSGGGGSHPIPDSSPLLQFGGQVRQVYLYTDDAQQTEAHLEIREDGTVGGAADQSPESLLQLKALKPGVIQILGVKTSRFLCQRPDGALYGSLHFDPEACSFRERLLEDGYNVYQSEAHGLPLHLPGNKSPHRDPAPRGPAVFLPLPGLPPALPEPPGILAPQPPDVGSSDPLHMVGGSQGLSPSYAS

SEQ ID NO: 4 - protein, 470 aa, synthetic construct
HGEGTFTSDVSSYLEEQAAKEFIAWLVKGGGGGGGSGGGGSGGGGSESKYGPPCPPCPAPEAAGGPSVFLFPPKPKDTLMISRTPEVTCVVVDVSQEDPEVQFNWYVDGVEVHNAKTKPREEQFNSTYRVVSVLTVLHQDWLNGKEYKCKVSNKGLPSSIEKTISKAKGQPREPQVYTLPPSQEEMTKNQVSLTCLVKGFYPSDIAVEWESNGQPENNYKTTPPVLDSDGSFFLYSKLTVDKSRWQEGNVFSCSVMHEALHNHYTQKSLSLSLGGGGGSGGGGSGGGGSHPIPDSSPLLQFGGQVRQVYLYTDDAQQTEAHLEIREDGTVGGAADQSPESLLQLKALKPGVIQILGVKTSRFLCQRPDGALYGSLHFDPEACSFRERLLEDGYNVYQSEAHGLPLHLPGNKSPHRDPAPRGPARFLPLPGLPPALPEPPGILAPQPPDVGSSDPLHMVGGSQGLSPSYES

SEQ ID NO: 5 - protein, 470 aa, synthetic construct
HGEGTFTSDVSSYLEEQAAKEFIAWLVKGGGGGGGSGGGGSGGGGSESKYGPPCPPCPAPEAAGGPSVFLFPPKPKDTLMISRTPEVTCVVVDVSQEDPEVQFNWYVDGVEVHNAKTKPREEQFNSTYRVVSVLTVLHQDWLNGKEYKCKVSNKGLPSSIEKTISKAKGQPREPQVYTLPPSQEEMTKNQVSLTCLVKGFYPSDIAVEWESNGQPENNYKTTPPVLDSDGSFFLYSKLTVDKSRWQEGNVFSCSVMHEALHNHYTQKSLSLSLGGGGGSGGGGSGGGGSHPIPDSSPLLQFGGQVRQVYLYTDDAQQTECHLEIREDGTVGCAADQSPESLLQLKALKPGVIQILGVKTSRFLCQRPDGALYGSLHFDPEACSFRERLLEDGYNVYQSEAHGLPLHLPGNKSPHRDPAPRGPARFLPLPGLPPALPEPPGILAPQPPDVGSSDPLHMVGASQGLSPSYAS

SEQ ID NO: 6 - protein, 470 aa, synthetic construct
HGEGTFTSDVSSYLEEQAAKEFIAWLVKGGGGGGGSGGGGSGGGGSESKYGPPCPPCPAPEAAGGPSVFLFPPKPKDTLMISRTPEVTCVVVDVSQEDPEVQFNWYVDGVEVHNAKTKPREEQFNSTYRVVSVLTVLHQDWLNGKEYKCKVSNKGLPSSIEKTISKAKGQPREPQVYTLPPSQEEMTKNQVSLTCLVKGFYPSDIAVEWESNGQPENNYKTTPPVLDSDGSFFLYSKLTVDKSRWQEGNVFSCSVMHEALHNHYTQKSLSLSLGGGGGSGGGGSGGGGSHPIPDSSPLLQFGGQVRQVYLYTDDAQQTECHLEIREDGTVGCAADQSPESLLQLKALKPGVIQILGVKTSRFLCQRPDGALYGSLHFDPEACSFRERLLEDGYNVYQSEAHGLPLHLPGNKSPHRDPAPRGPARFLPLPGLPPALPEPPGILAPQPPDVGSSDPLHMVGGSQGLSPSYAS

SEQ ID NO: 7 - protein, 470 aa, synthetic construct
HGEGTFTSDVSSYLEEQAAKEFIAWLVKGGGGGGGSGGGGSGGGGSESKYGPPCPPCPAPEAAGGPSVFLFPPKPKDTLMISRTPEVTCVVVDVSQEDPEVQFNWYVDGVEVHNAKTKPREEQFNSTYRVVSVLTVLHQDWLNGKEYKCKVSNKGLPSSIEKTISKAKGQPREPQVYTLPPSQEEMTKNQVSLTCLVKGFYPSDIAVEWESNGQPENNYKTTPPVLDSDGSFFLYSKLTVDKSRWQEGNVFSCSVMHEALHNHYTQKSLSLSLGGGGGSGGGGSGGGGSHPIPDSSPLLQFGGQVRQVYLYTDDAQQTEAHLEIREDGTVGGAADQSPESLLQLKALKPGVIQILGVKTSRFLCQRPDGALYGSLHFDPEACSFRERLLEDGYNVYQSEAHGLPLHLPGNKSPHRDPAPRGPARFLPLPGLPPALPEPPGILAPQPPDVGSSDPLHMVGASQGLSPSYES

SEQ ID NO: 8 - protein, 470 aa, synthetic construct
HGEGTFTSDVSSYLEEQAAKEFIAWLVKGGGGGGGSGGGGSGGGGSESKYGPPCPPCPAPEAAGGPSVFLFPPKPKDTLMISRTPEVTCVVVDVSQEDPEVQFNWYVDGVEVHNAKTKPREEQFNSTYRVVSVLTVLHQDWLNGKEYKCKVSNKGLPSSIEKTISKAKGQPREPQVYTLPPSQEEMTKNQVSLTCLVKGFYPSDIAVEWESNGQPENNYKTTPPVLDSDGSFFLYSKLTVDKSRWQEGNVFSCSVMHEALHNHYTQKSLSLSLGGGGGSGGGGSGGGGSHPIPDSSPLLQFGGQVRQRYLYTDDAQQTEAHLEIREDGTVGGAADQSPESLLQLKALKPGVIQILGVKTSRFLCQRPDGALYGSLHFDPEACSFRERLLEDGYNVYQSEAHGLPLHLPGNKSPHRDPAPRGPARFLPLPGLPPALPEPPGILAPQPPDVGSSDPLHMVGASQGLSPSYAS

SEQ ID NO: 9 - protein, 470 aa, synthetic construct
HGEGTFTSDVSSYLEEQAAKEFIAWLVKGGGGGGGSGGGGSGGGGSESKYGPPCPPCPAPEAAGGPSVFLFPPKPKDTLMISRTPEVTCVVVDVSQEDPEVQFNWYVDGVEVHNAKTKPREEQFNSTYRVVSVLTVLHQDWLNGKEYKCKVSNKGLPSSIEKTISKAKGQPREPQVYTLPPSQEEMTKNQVSLTCLVKGFYPSDIAVEWESNGQPENNYKTTPPVLDSDGSFFLYSKLTVDKSRWQEGNVFSCSVMHEALHNHYTQKSLSLSLGGGGGSGGGGSGGGGSHPIPDSSPLLQFGGQVRQRYLYTDDAQQTEAHLEIREDGTVGGAADQSPESLLQLKALKPGVIQILGVKTSRFLCQRPDGALYGSLHFDPEACSFRERLLEDGYNVYQSEAHGLPLHLPGNKSPHRDPAPRGPARFLPLPGLPPALPEPPGILAPQPPDVGSSDPLHMVGGSQGLSPSYAS

SEQ ID NO: 10 - protein, 470 aa, synthetic construct
HGEGTFTSDVSSYLEEQAAKEFIAWLVKGGGGGGGSGGGGSGGGGSESKYGPPCPPCPAPEAAGGPSVFLFPPKPKDTLMISRTPEVTCVVVDVSQEDPEVQFNWYVDGVEVHNAKTKPREEQFNSTYRVVSVLTVLHQDWLNGKEYKCKVSNKGLPSSIEKTISKAKGQPREPQVYTLPPSQEEMTKNQVSLTCLVKGFYPSDIAVEWESNGQPENNYKTTPPVLDSDGSFFLYSKLTVDKSRWQEGNVFSCSVMHEALHNHYTQKSLSLSLGGGGGSGGGGSGGGGSHPIPDSSPLLQFGGQVRQQYLYTDDAQQTEAHLEIREDGTVGGAADQSPESLLQLKALKPGVIQILGVKTSRFLCQRPDGALYGSLHFDPEACSFRERLLEDGYNVYQSEAHGLPLHLPGNKSPHRDPAPRGPAQFLPLPGLPPALPEPPGILAPQPPDVGSSDPLHMVGGSQGLSPSYAS

SEQ ID NO: 11 - protein, 470 aa, synthetic construct
HGEGTFTSDVSSYLEEQAAKEFIAWLVKGGGGGGGSGGGGSGGGGSESKYGPPCPPCPAPEAAGGPSVFLFPPKPKDTLMISRTPEVTCVVVDVSQEDPEVQFNWYVDGVEVHNAKTKPREEQFNSTYRVVSVLTVLHQDWLNGKEYKCKVSNKGLPSSIEKTISKAKGQPREPQVYTLPPSQEEMTKNQVSLTCLVKGFYPSDIAVEWESNGQPENNYKTTPPVLDSDGSFFLYSKLTVDKSRWQEGNVFSCSVMHEALHNHYTQKSLSLSLGGGGGSGGGGSGGGGSHPIPDSSPLLQFGGQVRQQYLYTDDAQQTEAHLEIREDGTVGGAADQSPESLLQLKALKPGVIQILGVKTSRFLCQRPDGALYGSLHFDPEACSFRERLLEDGYNVYQSEAHGLPLHLPGNKSPHRDPAPRGPAQFLPLPGLPPALPEPPGILAPQPPDVGSSDPLHMVGASQGLSPSYAS

SEQ ID NO: 12 - protein, 470 aa, synthetic construct; identical to SEQ ID NO: 7